European Patent Specification EP 3 697 930 B1, published July 12, 2023. Title: PRIMER-INDEPENDENT DNA POLYMERASES AND THEIR USE FOR DNA SYNTHESIS. Applicant: Consejo Superior de Investigaciones Científicas (CSIC) Pasteur Institute. The sequence listing filed with the application follows.

SEQUENCE LISTING (85 sequences)

SEQ ID NO: 1 - protein, 14 aa, Artificial Sequence
  Common conserved domain within the piPolBs described in the invention, needed for priming activity
  MISC_FEATURE (2)..(2): A, H, K, T, D, Y, G or R
  MISC_FEATURE (3)..(10): Any amino acid
KXXXXXXXXXKTRG

SEQ ID NO: 2 - protein, 866 aa, Escherichia coli
MSNNLQDILAAASGYQSVTSEPALNRKRPKTLDDYPVIPPASKKVSVISSDLTLHIGFDTEYVFNPETRQNDILSYQSYVVLPDNTGISNIIYPPDSQKKSRLSFKDFLCQTITPLLETGVITKWPGIINIYAHFIRADIASFANFWSDYKILLKGIRGTVSSFKNRYGIDFDEQQERRVKTEQIMFDKRTSPPRCSNVAFIDTLLITPGGMGLAECGELLGLPKLTIPAPYSITNMREYLLGDRAGFEAYALRDAEIAVRYALQVRNFCARELMIDRVPATIGAMAVSRFTKTLKENNMSPEVCLGTHIKTRELWLTEKQAFRTIKNPASVPSRELFETFPINCYHGGRNECFMMGVTPSDHWYDYDLAGAYTTGLLDILTPDYGNIRLSKNPDDYCGHVMGFALVTFRFPESVPYPSLPVRTDQYGLFFPLSGESWATAPEIELALSLGAEMTIHNGIIVPWICDTSPHNSESTSVFLPFVQQVRENRNRHIKGSLEEKFWKEIGNSLYGKLAQGLRAKTAFDTARGLNRSLPPSSVTQPFFAAHVTGFIRAVVGELMNALPSDSSVVSVTTDGFLTNCPLDKINMSGPLSSRFQSLCDIVDPGSSMLTCKHEVSQLIAMKTRGQLTYKAIQGKPVVHARAGVKPPADIPRSDYNDYMVDLYLNRLPGQTLSRSTLISTREMWLSESDLVSREQDIRLNLEFDFKRQPVRPAMNEGHLLMFSRPWDNMEEALQQRSLFDDWRQTHTLKTLADWDDWCDFLYCRTVFSDMKLKVGSKRSDDILVRLFLRALTQCQWGLMLKDKKSYSCKEVAEWLTSEGYSVTVTDVKNAVRAKIPQMKFSSVTPRMKSLMDIIARKYPTFCLPV

SEQ ID NO: 3 - protein, 586 aa, Artificial Sequence
  Parental DNA pPolB of phi29 (SEQ ID NO: 6) comprising its KxY motif substituted by SEQ ID NO: 1
  MISC_FEATURE (499)..(499): A, H, K, T, D, Y, G or R
  MISC_FEATURE (500)..(507): Any amino acid
MKHMPRKMYSCDFETTTKVEDCRVWAYGYMNIEDHSEYKIGNSLDEFMAWVLKVQADLYFHNLKFDGAFIINWLERNGFKWSADGLPNTYNTIISRMGQWYMIDICLGYKGKRKIHTVIYDSLKKLPFPVKKIAKDFKLTVLKGDIDYHKERPVGYKITPEEYAYIKNDIQIIAEALLIQFKQGLDRMTAGSDSLKGFKDIITTKKFKKVFPTLSLGLDKEVRYAYRGGFTWLNDRFKEKEIGEGMVFDVNSLYPAQMYSRLLPYGEPIVFEGKYVWDEDYPLHIQHIRCEFELKEGYIPTIQIKRSRFYKGNEYLKSSGGEIADLWLSNVDLELMKEHYDLYNVEYISGLKFKATTGLFKDFIDKWTYIKTTSEGAIKQLAKLMLNSLYGKFASNPDVTGKVPYLKENGALGFRLGEEETKDPVYTPMGVFITAWARYTTITAAQACYDRIIYCDTDSIHLTGTEIPDVIKDIVDPKKLGYWAHESTFKRAKYLRQKXXXXXXXXXKTRGIQDIYMKEVDGKLVEGSPDDYTDIKFSVKCAGMTDKIKKEVTFENFKVGFSRKMKPKPVQVPGGVVLVDDTFTIK

SEQ ID NO: 4 - protein, 746 aa, Artificial Sequence
  Parental DNA pPolB of Bam35 (SEQ ID NO: 7) comprising its KxY motif substituted by SEQ ID NO: 1
  MISC_FEATURE (536)..(536): A, H, K, T, D, Y, G or R
  MISC_FEATURE (537)..(544): Any amino acid
MMTTTNRKKRREIKLFTLDTETRGLDGDVFRIGLFDGKQYYTGYTFADVLPVFEKYKAYDCHVYIHNLDFDLSKIIAELRDYAEPTFNNSLFINGNIVTFTASHIILHDSFRLLPSSLENLCRDFDLLEGGKMDIVDYMEENNYGIYNVKNRKLNKRLTKGNFFTTVDKDDPVLCEYMEYDCRSLYKILEIVIGLSKLEVEQFINCPTTASLAKTVYKEQYKKDYKVAISTKQYNHKQIGKGLEAFIRKGYYGGRTEVFTPRIENGYHYDKNSLYPYVMKMAEMPVGYPNVLDNEEAELSFDLWKRRKYGAGFIHAKVHVPEDMYIPILPKKDYTGKLIFPVGKIEGVWTFPELALAEAEGCRIEKIESGVVFEKTAPVFREFISYFEEIKNTSKGAKRAFSKLMQNALYGKFAMQRERIMYADISERDKLEAEGHTVSEIIYDMNGIRMEFLEYDGYAKAEYIQPHISAYITSIARILLFKGLKYAHEKGILAYCDTDSCATTTKFPDKMVHDKEYGKWKLEGYVIEGLYFQPKXXXXXXXXXKTRGAEKAINTDGEYEEVLRMKGVPKWVVEEQLDYNTFKKWYLQVKRGKAEIPIYKGGERVQKFLTKSKNNIEMNELAEMHKTINFAREQKRNIDLNKNTTSPLVRNDYGENKDEKSEYEFDEWYERLEEFNDDMNAVEELCMKFGKIQIPEKKQRKLYGLYKEYSSKAKAMCFSNEGLPIQDWCKKTGWDMKELLGELSFL

SEQ ID NO: 5 - protein, 8 aa, Artificial Sequence
  X3-10 amino acid sequence within SEQ ID NO: 1
EVSQLIAM

SEQ ID NO: 6 - protein, 575 aa, Phage phi29 [sequence omitted]

SEQ ID NO: 7 - protein, 735 aa, Phage Bam35
MMTTTNRKKRREIKLFTLDTETRGLDGDVFRIGLFDGKQYYTGYTFADVLPVFEKYKAYDCHVYIHNLDFDLSKIIAELRDYAEPTFNNSLFINGNIVTFTASHIILHDSFRLLPSSLENLCRDFDLLEGGKMDIVDYMEENNYGIYNVKNRKLNKRLTKGNFFTTVDKDDPVLCEYMEYDCRSLYKILEIVIGLSKLEVEQFINCPTTASLAKTVYKEQYKKDYKVAISTKQYNHKQIGKGLEAFIRKGYYGGRTEVFTPRIENGYHYDKNSLYPYVMKMAEMPVGYPNVLDNEEAELSFDLWKRRKYGAGFIHAKVHVPEDMYIPILPKKDYTGKLIFPVGKIEGVWTFPELALAEAEGCRIEKIESGVVFEKTAPVFREFISYFEEIKNTSKGAKRAFSKLMQNALYGKFAMQRERIMYADISERDKLEAEGHTVSEIIYDMNGIRMEFLEYDGYAKAEYIQPHISAYITSIARILLFKGLKYAHEKGILAYCDTDSCATTTKFPDKMVHDKEYGKWKLEGYVIEGLYFQPKMYAEKAINTDGEYEEVLRMKGVPKWVVEEQLDYNTFKKWYLQVKRGKAEIPIYKGGERVQKFLTKSKNNIEMNELAEMHKTINFAREQKRNIDLNKNTTSPLVRNDYGENKDEKSEYEFDEWYERLEEFNDDMNAVEELCMKFGKIQIPEKKQRKLYGLYKEYSSKAKAMCFSNEGLPIQDWCKKTGWDMKELLGELSFL

SEQ ID NO: 8 - protein, 965 aa, Acidithiobacillus caldus SM-1
MRGPVPRRQGGEGTVAILAMTLHEASCSAVGIQPQPCTATAAIAEPSCPALLPEPTAAVTQPQRDAPCQDLSNANTAVPFSSYRFESQMETEFGPLRLYVFRGQKAKESIQVDDEYTSDYSQHIDNTSTSAGVITSMGPDEGIDTNGNDQTRLVVALDAEWQESEGQAGGETQKRKILCLQAATRFRDGTRVVCLLYLRSRRRPSQGQFLQLLWGQWQRLGLVPALVYRPKPKPTSDSTDRKCCTAVKTQALLYLVGHYGIVDNTSFYNRRKIVQNADAVRRTIVSVQYPTSVYFYDRGRRRAKVTVFYRDTMLLSPSGSSLEMLGDALDFPKIQLPEGYKKSDMRQFLKEKPLQFEEYAATDALIALEWIFRNSWGREVPITLGGEGARLFRDHIMTARGWTIDEFDFHLRGLARKIIDTGEGKRIKKKEPRSNTTTLIARATESYYGGRNECILSGIHHGPWYDFDIAGAYPAAMSLIPDPDYDQPRITLLPGPLPREMIRPEMLLFAHVSFTFPDEIRYPCLPIKDSSGRGLIFPRSGETWAAAPELWLAQRWGAEITLLEPTEIIPTRNTFSLADGMRAMVQERERLKSRFGKKSIEQTRQKEMNNSVYGKLAQGLSGKRSYSPRADRTEEVGPSILTCAPLAALTTAWVRALVSAMMQSLHVAGYRVASVTTDGFLCDAHSLDGLTTWGIAEAFIDGRKRLGLDSNLWELKHAAQSLVMMKTRGGYGLGRVGDLPLPIARAGYKSSQEDTSEALARVYLERRGRVVTEEVRLPTMREYVRHEADGTGRIQRKELSLDYDFKRCPQKIWTETIVIQGQSYEHVSFDSVPWGSIDEFTNAREVIDQHHDTPLKSESDLKQALLRVERHTAVKSVGLRVNNNVAISGAVSVLRGLRAGGISAPWFDPDVTSGKTVLERVGAVFGVKLSTNDWKNAGRKERQKQGWSLIGFDREVAALELTEKT

SEQ ID NO: 9 - protein, 864 aa, Colwellia sp. MT41
MFNEDEGYPSITSETQLSYEEPSSVAVPIPFDENKLNTYGSSAQNKSQREKKVPIQMRPVLGFDTEYHRSSDNTYNVILSYQSYLFNPVNGRSCKAVFYPSKRSKDGRIGIKKFITLVIEDALKQGVLTDIPRDIFGCAHFLRADFSSFKNAFSDMKDSIKGLRNSVASLGETYGVDIDAIDAKKVSNLSTTYWDKNRNSHPIQLAFYDTMFFAPAGKTLKDVGEFVGREKLEIPEPYSIDKMDVFLKEEKVLFEEYGIRDAEISALHLLRTLQLCASLGLKGLPYTIGGIAVKVFMAKLGTKARYLELFALEEYKVERWSKTKNTPVTSTKNLLKASASFDEHLASKCYHGGRNEAFFTGPTPVLPWFDVDLKSCYSIAVSNLRPLDHENRFHTKDINDFSGDVFGLAWVEFEFPTSVQYPTLPVRTDSDMLVFTQKGFSYCTAQEIDVSRRLGVKIVIKEGLIIPWLNDDYFCVPFMHSMRAERNKAEKGSFEDRMFKELSNTLYGKIAQGVKSKTSFEISSGLSKPVSPSVVTNPYFAAYITGLARAVIGDMINAIPTPYSVLSVTTDGFITDAPLTEIPIDSPVCNLFRESYHRMDDTGGDILEEKHRVNQLLVLKTRGQLTLKPCDGHPSIIAKAGVKTPNNCKDQNAYMVDLYLNRTPQTKTDASHLTATRPQFIGQQDLMMVPKMCRLNLEPDLKRKLLPPIEVEVNGVKHVAMGSVPYEDLQTLEQDRLFFTRWRANNNMKTLADYASWDEFVKLRRTKNLKGVNLKVDETADAFLVRLFLRVIAQEQFGVTLGYGVKPNAISSAKKAKVITGAVPLTANVIKVLKLILIIFPDFDYQAMIAPEYHLELKQLMSSI

SEQ ID NO: 10 - protein, 902 aa, Vibrio parahaemolyticus
MEENMNYWAEDSGVEIEESFDGIEVDESLVEAWGNASNDDHVDETLGSISEETKPLVENINEYENSKKKSKRYKARTKFFDRPIISFDTEYVLSKCGKYNRVLSYQFVTLHNGKVSKLVLYPDSAKKSGRLSMDYCFARVIEKAIEDDVLERWPTDIIVTAHFMKADLFNFNQAFEQIKTHIKGIRKTVASLGGAYELDLSKVMTRRIDKEPVQIKDKNRNYHTLHMSFFDTMLLAPASAQSLSAVGNIVGVPKLEIPEPYSIERMDEYLAGNKTGFEAYGLTDSLISALHFKATADLCKELGLKSVPYTIGGMAVKTFINSLDDPKSYRKLFGFEEEKREIWSKETGKVRTVTIEEPTQARKTMEWFASECYSGGRNEAFWSGVTPVDTWLDLDVPSCYSAITNGLREISYEDMYMSNEVEDFFGDKMALAWVEFEFPSSTRHPSLVVRDKDSLIFPLRGETHCTGHELEVAYNQGAKIKIKQGFIFPWKNDVRIFEKYMKWGREKRKSYEKGSFQEKLVKEMLNSTYGKFSQNVKPKQTFSVEDGYSKPQPPSKLTNPFYASYTCGLARALLGEMLSGVPSNKTVVSVTTDGFLTNADIEEIDLSGPICQRFRELFHRMEPNGGEILEVKHKAKQLICAKTRAQYTVTPMEGWEPVLAKGGVQVPKQVTDQNQYMVDLYKERTPEHMTDSSHLTSLRSMCTERKDMLMERKQSRLNLEFDMKREPINPRVIEVDGVPLVSFETKPFKNAFEMRYTRIRFDAWRKSGRCLKTMDDWYDWQERLSMYKANDKGEVRLKKDEKSDELMARLFVRFYGHEASGITKKDITAKALSEWLVELGYDIKPSLVRGAGRTKLVEGTVPLTPSTLKLAKLLMDKFPQFDPVPLFNASDEEVMRQLENIS

SEQ ID NO: 11 - protein, 911 aa, Vibrio parahaemolyticus
MEENMNVWAQSVELEINEELTFSDVEADFTSAWGSSDELLNEYAEDEKQSLADAVVETASPIDSEALKAWTEPKKKGQRRIGTKFYDRPIIGFDTEFELSKCKKYNHVISYQLVVRHKGRTSKLVLYPDSNKKSGRLAMDYCLARVIEKAIEDGTLERWPTDVIMTAHFMKADLFHFNKAFDQVKTHIKGIRKTVASLGDAYALDLSKVLSRRIDEEPVDVYDKNRNKKTLHLSFFDTMLLAPAGKSLADVGELVGLTKLKIPEPYSIERMGEYLTGNKQGFEAYGLRDAELSALHFEKTANLCKELGLKSVPYTIGGMAVKAFINSLDDPKNYRKLFGFEKKTFEVWSKDQAKVKTVTVDEPTPARSTMEWFASECYSGGRNEAFWASATHIDTWNDLDVPSCYTAITNALRPIAYDRMYMSNRVEDFFGDKMALAWVEFEFPPQTRFPSLVVRNKDSLIFPLSGETHCTGHELEVAYNQGAKITIKQGFIFPWASEERIFEKYMLWGRQKRKSYPKNSYQEKLIKEMLNSTYGKFSQNVKPKKTFSVADGYSQPQQPSKLTNPFYASFTCGMGRALLSEMLAGVPDDKTVVSVTTDGFLTNAKIEEIDLSGPVCQRFRELFHRMEPNGGEILEIKHKAKQLICAKTRAQFTVIPEEGWEPVLAKGGVRPPEGEVDHNRYMVNLYKERTPEHTVDTSHLTSLRVMCTEGQDMKMERKESRLNLEFDMKRELIKPIMVDIEGQPNVSFDSKPFKNAFEMRYTRIRFDAWRKSGHCLKTLEDWYDWQERLRMYKAKDKAMSNDNCKVRFKKDEKADELMARLFVRFYGHEASGISKKDITAKALSEFLVGLGYEIKPSLVRGAGRTELVEGVVPLMHSTMQLAKQLVERFPQFDPTPLFDVDDAEELKHSLK

SEQ ID NO: 12 - protein, 892 aa, Moritella sp. PE36
MINELMVWEQDESTVSELSNEDTGLSSTWDEDNLSDNEAMLSVAEYEVSHSITKGKGKDKAKKGKRRVGTKFFERPTVSLDTEYTESPCGTYNRILSYQFVVRHEGKSSGIILYPESTKKSGRLALDKCLVLALEKAMAEDVLTCWPTDIILVAHFLKADLFNFSNAFDQLKTHVKGLRKTVASLDEPYGLDLDEVLSRRIDKEPLEVYDKTRNYHTLYITFYDSMLLSPNGKSLADVGRLVGLPKLDIPAPYSISRMDEYRDADPEGYAAYAMNDGFVTSLHFERISKFCKDIGLKSVPFTIGGIAVKAFVNGLADSKGYRQLFGFMKVTKEVWPEDRNKPLTLTRDVPVTARMTLENFATQAYSGGRNESFIAGSVPIDTWNDFDAPSCYTAICLGLRKLAYDRMFMTKKLEDLFGDKCALAWVRFEFPASTRFPSLAVRSDKGLIFPLTGETHCTGHELEVASNQGAIITIKQAFVIPWADDVRIFENFMGWVRENRQANVKGGFEERLFKEIGNTLYGKFSQSLRPKTAFDIQAGYSKQLPPSTLTNPFFAAYTTGLARALMGEMVASIPDHRTVVSLTTDGMATNATLEEFDLNGPICQRFREHFHRIDPNGGEILELKHQAKQLIGAKTRAQYTVLESEGFAPILAKGGVMVARSVVNQSAYMVDLYLNRHVGQLTDGSHLTSTREMFIGRKDMMNEQREILLNMEYDHKRELIDPVMIDVKGQRHISLQSKPHHSLDDMLFTRLRFDRWRKNNCLKTMDDWITWHDRLAMAKASKNKSVNLKKDETSGEYMARLFLRFYGYEHAGIRKSDINATQLALWLTEQGYPTKAAAVRGAGRSDLVEGAVPLTELTIKFAKLLVAKFPNFNPERLFEASSRPQLREALKQ

SEQ ID NO: 13 - protein, 904 aa, Vibrio cyclitrophicus
MSETYDWLEQDTSITIGNLTETGWEECDVESEDSWEAQESVDVKDVPFKTVKPKVKPYIGKKPPKKVKVKRKKRKATPFFERPVIAIDTEYTESDCGEYNSILSYQLAILHKGLLSTLILYPESTKKSGRLALDRCLVQAIEKAMDEGVLDTFPTDVILCAHWLSADLFNFSKAFDQLKTHVNGLRKTVASLDDVYGLELDKVMSRRIDKEPLQVNTKSRNKKTLYITFFDTMLLSPNGSSLSSVGDLLEIPKVEIPEPYSISRMDEFLEAEPEKFAEYALTDAIISARHFERVSLFCQHTLGLKSVPFTIGGIAVKAFVNSLEDKRGYRGLFGFEKVTKEIWPSDRNKPLTITRDVPVTARMTLENFATQCYHGGRNESFIAGPTQVDTWRDYDIPSCYSAITLGLRELAYEKMYMTEDLHDLFGDKCAMAWVEFKFPENTRFPSLAVRSDYGLLFPITGETYVTGHELEVAYNQGAEITIKQAFVIPWKNDVRIFEDFMKWGRERRKSFVKGSFDERLTKEMLNSCYGKMAQSLRPKSAFDIQAGYSKQLPPSTLTNPFFAAYITGLARAYLSFLIHSVPANKTVISSTTDGFLTNASLDEIDLTSPICQRFRDLYHRIDPSGGEILELKHQAKQLIGAKTRAQYTVIESDGFEPVLAKGGIKVDPTIVDQSAHMVDKYIDRSFDDKVDGSYLTPNRMRFLEHKDLMLEKRSIFLNMEYDQKRELMNPKMLDVKDRQHIALETKPHYSLGDMLFTRLRFDHWRKQHCLKTLEDWYNWQDRLAMAKASNNKSLRLKSDETSDSLMARLFLRFYAHEQGGISKSDINANQLASWLTEQGYPTKSTLVRSAGKSKLIEAAVPLTELTIKLAILIKSKFPSFEIEKLFEPIARESLRAALSSQLSS

SEQ ID NO: 14 - protein, 903 aa, Vibrio jasicida
MEESMNNWGEDAGVEIDESFDGIEVDENLVEAWGNASNDELLDESVGSIVFERMQPVEKVSEYVKSKKEKKKKEKRKATPFFERPVIAMDTEYVESECGTYNRILSYQFAVLYKGKLSTTILFPESTKKLGRLALDKCLVQAIEKAMDDEVLDRWPTDIILCAHWLSADLFNFSQAFEQLKTHVKGLRKTVASLDDVYGLDLENVMSRRIDKEPLQTYSKSGNKKTLYITFYDTMLLAPNGQSLASVGKILKVPKVEIPEPFSISRMDEFLAAEPEQFAEYAITDAIISARHFERVSSFCQQTLGLKSVPFTIGGIAVKAFVNSLEDKRSYRGLFGFEKVTKEVWPSDRTKPLTLTRDVPVTARMTLENFATQCYHGGRNESFIAGPTVIDTWRDYDVPSCYSAITLGLRELAYEQMYMTKDLNDLFGDKCAMAWVEFKFPERTRFPSLAVRSDYGLVFPLTGVTHCTGHELEVAKNQGAEITVKQAFVIPWANDERIFEPFMKWGRERRKSFDKGSFDEKLTKEMLNSCYGKLAQSLRPKTAFDIQAGYSKQLPSSTLTNPFFAAYTTGLARALLGEMLHSIPDDKVVVSVTTDGFLTNATLDEIKLDGVICQRFRDLYHRIDPSKGKVLELKHQATQLIGAKTRAQYTVIKSEGYEPILAKGGVKVDPMVTDQSAYMVNKYLERQPDDKVDGSYLTPNRIRFLEQKDLMLEKRSIFLNMEYDQKRELVNPKMIDVKGKQHIALETVPHQSLDSMSFTRIRFDHWRKNHCLKSMGDWHDWQERLSMYKANDKREIRLKKAEKSDELMARLFVRFYGHEVSGITKKDITAKALSDWLVSLGYDIKPSLVRGAGRTKLVEGVVPVTHSTLKLTKLLVGKFPQFDPVPLFNSSREEIMRQLENIS

SEQ ID NO: 15 - protein, 897 aa, Vibrio sp. J2-4
MNETYSWLEQDSNLKMDTLAASGWMEDDPVSTWMKPQSDVSEPDLGVKRKAKPILLRKPKKKKQTKRKKRKATPFFERPVVAIDTEYRESEDETYNRIISYQVAVLFRGKLSTIILYPESTKKSGRLALDKCLVQAIEKAMDEGVLDAWPTDIILCAHWLSADLFNFSQAFDQLKTHVKGLRKTVASLDDVYGLELDKVMSRRIDKEPLQVRTKTRNPKTLYITFYDTMLLSPNGSSLASVGELLKVPKVEIPEPYSISRMDEFLEAEPEMFAEYAITDAIISARHFERVSAFCQHTLGLNSVPFTIGGIAVKAFVNSLEEQQGYRGLFGFEKVTKEVWPSDRTKPLTITRDVPVTARMTLENFATQCYHGGRNESFIAGPSVIDTWRDYDVPSCYSAITLGLRELAYDQMYMTKDLHDLFGDKCALAWVEFKFPENTRFPSLAVRSEYGLIFPLSGETHCTGHELEVAYNQGVEITIKQAFVVPWKNDERIFESFMKWGRERRKSFVKGSFDEKLTKEMLNSCYGKLAQSLRPKNSFDIQAGYSKQLPPSTLTNPFFAAYTTGLARALLGEQLHSIPDDKVVVSVTTDGFLTNAELDEIDLSGSICQRFRELYHRIDPTGGEVLELKHQATQLIGAKTRAQYTVIESEGFEPVLAKGGVKVDPTITDQSAYMVEKYLARKPGDKVDGSYLTPNRMRFLEHKDLMLEKRSIYLNMEFDQKREMLNPVMVDVQGRQHIALETKPHQSLDEMLFTRLRFDRWRKSHVLKDFDDWCSWQDRLVMAESTSHKDVRLKADETSDSLMARLFLRFYAHEKNGMRKKDITAKALAEWLTDLGYPTKATAVRSAKQSKLIEGAVPITELTTNLARLIVSKFPDFEVEILFNPDSRSSLREALSVN

SEQ ID NO: 16 - protein, 897 aa, Vibrio parahaemolyticus NBRC 12711
MSKNFNWLEQSSDLSMDNLATSGWTEEEAVSAWGEAQPSEPASFDGVKRKAKSIVLRKPKKKKQTKRKKRKATPFFERPVIAMDTEYVVSKCGGYNRILSYQFAVLFQGKLSTIILFPESTKKSGRLALDKCLVQAIEKAMEDEVLDKWPTDIILCAHWLSADLFNFSQAFDQLKTHVKGLRKTVASLDDVYGLELDKVMSRRIDKEPLQAYSKSGNKKTLFITFYDTMLLSPNGSSLASVGELLKIPKVEIPEPYSISRMDEFLEAEPEKFAEYAITDSIISARHFERVSSFCQNTLGLNSVPFTIGGIAVKAFVNSLEDKRGYRGLFGFEKVTKEVWPSDRSKPLTITRDVPATARMTLENFATQCYHGGRNESFIAGPTGIDTWRDYDVPSCYSAITLGLRELDYDQMYMTKDLNDLLGDKCALAWVEFKFPEHTRFPSLAVRSEYGLIFPLSGETHCTGHELEVAYNQGAEITIKQAFVVPWKNDKRIFEDFMRWGRERRKSFVKGSFDEKLTKEMLNSCYGKLAQSLRPKRSFDIQAGYSTQLPPSTLTNPFFAAYTTGLARALLGEMLHSIPDDKVVVSVTTDGFLTNAELHEIDLKGPICQRFRELYHRIDPTGGEVLELKHQAKQLIGAKTRAQYTVIESEGFEPILAKGSVKVDPMVTDQSAYMVNKYLTRKPGDKVDGSYLTPNRMRFLEHKDLMLEKRSIYQNMEFDQKRELLNPVMIDVQGSKHIALETKPHKSLDEMLFTRLRFDHWRKAHCLKTFEDWYDWQDRLVMAESTSHKDLRLKADETSDSLMARLFLRFYAQEQGGMSKKQISAKALAEWLTDNGYSTKANSVSRAMKAKLIEGAVPMTELTVNLARLIVSKFPDFEVEILFNPDSRSSLREALSPN

SEQ ID NO: 17 - protein, 897 aa, Vibrio furnissii NCTC 11218
MNENFDWLEQASDLSMDNLATSGWTEEEAVSAWGEAQPSEPTSFDSVKRKAKPLVGRKPKKKKQTKRKRREATPFFERPVIAMDTEYVESECGTYNRILSYQFAVLFEGKLSTIILLPESTKKSGRLALDRCLVQAIEKAMDDEVLDKWPTDIILCAHWLSADLFNFSQAFDQLKTHVKGLRKTVASLDDVYGLDLDKVMSRRIDKEPLNVHDKSRNRHTLYITFYDTMLLSPNGSSLASVGELLKIPKVEIPEPYSISRMDEFLEAQPQKFAEYSITDSIISARHFERVSAFCQHTLGLKSVPFTIGGIAVKAFVNSLEDKRGYRGLFGFEKVTKEVWPSDRSKPLTITRDVPATARMTLENFATQCYHGGRNESFIAGPTGIDTWRDYDVPSCYSAITLGLRELAYDQMYMIRDLNELFGDKCALAWVEFKFPEHTRFPSLAVRSEYGLIFPLSGETHCTGHELEVAYNQGAEITIKQAFVVPWKNDVRIFEPFMKWGRERRKSFTKGSFDEKLTKEMLNSCYGKLAQSLRPKRSFDIQAGYSTQLPPSTLTNPFFAAYTTGLARALLGEMLHNIPDDKVVVSVTTDGFLTNAELHEIDLKGPICKRFRELYHRIDPTGGEVLELKHQAKQLIGAKTRAQYTVIESEGFEPILAKGSVKVDPMVTDQSAYMVNKYLTRKPGDKVDGSYLTPNRMRFLEHKDLMLEKRSIYQNMEFDQKRQLLNPVMVDVKGRSHIALETKPHKSLDEMLFTRLRFDHWRKSHVLKDFDDWCSWQDRLVMAESTSHKMLRLKADETSDRLMARLFLRFYAQEQGGMSKKQITAKALAEWMTDIGYPTKATAVRSAKNAKLIEGAVPITELTINLARLIVSKFPDFEVEILFNPESRSSLREALYAR

SEQ ID NO: 18 - protein, 900 aa, Vibrio fluvialis
MNEKYDWLEQASDLSMDNLATSGWTEEEAVSAWGEAQPSEPASFDGVKRKAKSIVLRKPKKKKQTKRKKRKATPFFERPVIAMDTEYVESECGTYNRILSYQFAVLFEGKLSTIILFPESTKKSGRLALDRCLVQAIEKAMDDKVLDKWPTDIILCAHWLSADLFNFSQAFDQLKTHVKGLRKTVASLDDVYGLELDKVMSRRIDKEPLQAYSKSGNKKTLFITFYDTMLLSPNGSSLSSLSSVGDLLSIPKVEIPEPYSISRMDEFLEAQPEKFAEYAITDSIISARHFERVSSFCQNTLGLNSVPFTIGGIAVKAFVNSLEDKRGYRGLFGFEKVTKEVWPSDRSKPLTITRDVPATARMTLENFATQCYHGGRNESFIAGPTDIDTWRDYDVPSCYSAITLGLRELDYDQMYMTKDLNDLLGDKCALAWVEFTFPSTCRFPSLAVRSEYGLIFPLSGETHCTGHELEVAYNQGAEITIKQAFVVPWKNDVRIFEPFMKWGRERRKSFVKGSFDEKLTKEMLNSCYGKLAQSLRPKNSFDIQAGYSKQLPPSTLTNPFFAAYTTGLARALLGEMLHNIPDDKVVVSVTTDGFLTNAELHEIDLKGPICQRFRELYHRIDPTGGEVLELKHQAKQLIGAKTRAQYTVIESEGFEPILAKGSVKVDPMVTDQSAYMVNKYLTRKPGDKVDGSYLTPNRMRFLEHKDLMLEKRSIYQNMEFDQKRQLLNPVMVDVKGRSHIALETKPHKSLDEMLFTRLRFDHWRKAHCLKTSEDWYDWQDRLVMAETASNQNLRLKAKEASDSLMARLFLRFYAHEKSGMSKKQITAKALAEWMTDIGYPTKATAVRSAKNAKLIEGAVPMTELTINLARLIVSKFPDFEVEILFNPESRSSLREALNAR

SEQ ID NO: 19 - protein, 887 aa, Actinobacillus minor NM305
MLPNNVSSLKKDIPLRGDISLSDNPLLDILPNVLDHFSHNVGDEENEDEGKQPFIIALDSEYQLAEDGKRNIILSYQYVAATRDNQHSPIKGIIYTRRRKNGEEIRLRLKSFLRKVILDALQKNVITQFPKTVYVVAHFLRADLSSFLDFFQEKTIVQGIRKTLASITDTYGVDVDELLGKSHHKELVNLSDNNNNMKQISIRFIDTQLLTPAQQGLATLGEIVGLEKLSIPEPYSIERMEEYLKEDKQGFEAYALRDAEIVFLYAMKLLDFTESEFNRAYLPVTLASIGVSQFLDELKIQGIKSSSFLGMSEESKLTFNTNTGKYKRMKIKSLSGGALTLERFAIECYHGGRNEAFCCGYTPIETWYDYDLPSAYTTALINIHPLNYDGYFQTTNVNDFKGHTLGLARVEFRFPEDTRYPCLPVKTENGLIYPLSGISYCTAPEIEVALGLGCEIVILEGFVIPWETTDKTPFSSFVKFIRKKREMCISKESPNNMIAEISEKLWKEIGNSLYGKLAQGLKGKKTFDVAKGLNKLVPRSKITNAFYASYVTGFVRAVVSQLLSAIPPDKVAVSVTTDGFITNAHLSEFDLSSLSVVQRFSSLVKELTSDENRPVLELKHQVKQLCCMKNRGQFTVEADGEYPLILAKASVQVPDSLRQFGQSSAERRQVENSYIAELYFNREANQKVSRSTMISTRESFISQRDLIKIRSDIKLNLEFDMKRHFSVANSLIINNDERLFIQTKPWKDVQSFYHYRAIFDEWKIHHTLKKICDFHHWIEFSSAKVSAKGKRVNVSKTFGADKVLLRQFLRCFAKGVHGGRVDMTYKRLSKFLTEKGYTVSEVDIKNAARASAKIQEKSVARTPNTEKLLSVLLEIAPNFEAQRFFVT

SEQ ID NO: 20 - protein, 866 aa, Enterobacter hormaechei
MSHNLQDILAAASGYQSVTSEPALNLKRPKTLDDYPVIPPASEKVSVISSDLTLHIGFDTEYVFNPETQQNDILSYQSYVVLPENTGISNIIYPPDSQKKSRLSFKEFLCQTITPLLETGVITKWPGIINIYAHFIRADIASFANFWSDYKILLKGIRGTVSSFKNRYGIDFDEQQERRVKTEQIMFDKRTSPPRCSNVAFIDTLLITPGDMGLAECGELLGLPKLTIPAPYSITNMREYLLGDRAGFEAYALRDAEIAVRYALQVRNFCARELMIDRVPATIGAMAVSRFTKTLKENNISPEVCLGTHIKTRELWLTEKQAFRTIKNPASVPSRELFETFPINCYHGGRNECFMMGVTPSDHWYDYDLAGAYTTGLLDILTPDYGNIRLSKNPDDYCGHVMGFALVTFRFPESVPYPSLPVRTDQYGLFFPLSGESWATAPEIELALSLGAEMTIHNGIIVPWICDTSPHNSESTSVFLPFVQQVRENRNRHIKGSLEEKFWKEIGNSLYGKLAQGLRAKTAFDTARGLNRSLPPSSVTQPFFAAHVTGFIRAVVGELMNALPSDSSVVSVTTDGFLTNCPLNKINMSGPLSSRFQSLCDIVDPGSSMLTCKHEVSQLIAMKTRGQLTYRAIQGKPVVHARAGVKPPADIPRSDYNDYMVDLYLNRLPGQTLSRSTLISTREMWLSESDLVSREQDIRLNLEFDFKRQPVQPAMNEGHLLMFSRPWDNMEEAMQQRSLFDDWRQTHTLKTLADWDDWCDFLYCRTVFSDMKLKVGSKRSDDILVRLFLRALTQCQWGLMLKDKKSYSCKEVAEWLTSEGYSVTVTDVKNAVRAKIPQMKFSSVTPRMKSLMDIIARKYPTFCLPV

SEQ ID NO: 21 - protein, 866 aa, Escherichia coli ETEC H10407
MSNNLQDILAAASGYQSVTSEPALNRKRPKTLDDYPVIPPASKKVSVISSDLTLHIGFDTEYVFNPETQQNDILSYQSYVVLPDNTGISNIIYPPDSQKKSRLSFKDFLCQTITPLLETGVITKWPGIINIYAHFIRADIASFANFWSDYKILLKGIRGTVSSFKNRYGIDFDEQQERRVKTEQIMFDKRTSPPRCSNVAFIDTLLITPGGMGLAECGELLGLPKLTIPAPYSITNMREYLLGDRAGFEAYALRDAEIAVRYALQVRNFCARELMIDRVPATIGAMAVSRFTKTLKENNMSPEVCLGTHIKTRELWLTEKQAFRTIKNPASVPSRELFETFPINCYHGGRNECFMMGITPSDHWYDYDLAGAYTTGLLDILTPDYGNIRLSKNPDDYCGHVMGFALVTFRFPESVPYPSLPVRTDQYGLFFPLSGESWATAPEIELALSLGAEMTIHNGIIVPWICDTSPHNSESTSVFLPFVQQVRENRNRHIKGSLEEKFWKEIGNSLYGKLAQGLRAKTAFDTARGLNRSLPPSSVTQPFFAAHVTGFIRAVVGELMNALPSDSSVVSVTTDGFLTNCSLNKINMSGPLSSRFQSLCDIVDPGSSMLTCKHEVSQLIAMKTRGQLTYRAIQGKPVVHARAGVKPPADIPRSDYNDYMVDLYLNRLPGQTLSRSTLISTREMWLSESDLVSREQDIRLNLEFDFKRQPVRPAMNEGHLLMFSRPWDNMEEALQQRSLFDDWRQTHTLKTLADWDDWCDFLYCRTVFSDMKLKVGSKRSDDILVRLFLRALTQCQWGLMLKDKKSYSCKEVAEWLTSEGYSVTVTDVKNAVRAKIPQMKFSSVTPRMKSLMDIIARKYPTFCLPA

SEQ ID NO: 22 - protein, 887 aa, Escherichia coli E1520
MLLNLDSLCRDTAPGIFSELTMSNNLQDILAAASGYQSVTSEPALNRKRPKTLDDYPVIPPASKKVSVISSDLTLHIGFDTEYVFNPETRQNDILSYQSYVVLPDNTGISNIIYPPDSQKKSRLSFKEFLCQTITPLLETGVITKWPGIINIYAHFIRADIASFANFWSDYKILLKGIRGTVSSFKNRYGIDFDEQQERRVKTEQIMFDKRTSPPRCSNVAFIDTLLITPGGMGLAECGELLGLPKLTIPAPYSITNMREYLLGDRAGFEAYALRDAEIAVRYALQVRNFCARELMIDRVPATIGAMAVSRFTKTLKENNMSPEVCLGTHIKTRELWLTEKQAFRTIKNPASVPSRELFETFPINCYHGGRNECFMMGVTPSDHWYDYDLAGAYTTGLLDILTPDYGNIRLSKNPDDYCGHVMGFALVTFRFPESVPYPSLPVRTDQYGLFFPLSGESWATAPEIELALSLGAEMTIHNGIIVPWICDTSPHNSESTSVFLPFVQQVRENRNRHIKGSLEEKFWKEIGNSLYGKLAQGLRAKTAFDTARGVNRSLPPSSVTQPFFAAHVTGFIRAVVGELMNALPSDSTVVSVTTDGFLTNCPLDKINMSGPLSSRFQSLCDIVDPGSSMLTCKHEVSQLIAMKTRGQLTYRAIQGKPVVHARAGVKPPADIPRSDYNDYMVDLYLNRLPGQTLSRSTLISTREMWLSESDLVSREQDIRLNLEFDFKRQPVQPAMNEGHLLMFSRPWDNMEEALQQRSLFDDWRQTHTLKTLADWDDWCDFLYCRTVFSDMKLKVGSKRSDDILVRLFLRALTQCQWGLMLKDKKSYSCKEVAEWLTSEGYSVTVTDVKNAVRAKIPQMKFSSVTPRMKSLMDIIARKYPTFCLPV

SEQ ID NO: 23 - protein, 887 aa, Cronobacter sakazakii 696
MLLNLDSLCRDTAPGIFSELTMSHNLQDILAAASGYQSVTSEPALNRKRPKTLDDYPVMPPASKNVSVISNDLTLHIGFDTEYVFNPETRQNDILSYQSYVVLPDNTGISNIIYPPDSQKKSRLSFKEFLCQTITPLLETGVITKWPCIINIYAHFIRADIASFANFWSDYKILLKGIRGTVSSFKNRYGIDFDEQQERRVKTEQIMFDKRTSPPRCSNVAFIDTLLITPGGMGLAECGELLGLPKLTIPAPYSITNMREYLLGDRAGFEAYALRDAEIAVRYALQVRNFCARELMIDRVPATIGAMAVSRFTKTLKENNMSPEVCLGTHIKTRELWLTEKQAFRTIKNPASVPSRELFETFPINCYHGGRNECFMMGVTPSDHWYDYDLAGAYTTGLLDILTPDYGNIRLSKNPDDYCGHVMGFALVTFRFPESVPYPSLPVRTDQYGLFFPLSGESWATAPEIELALSLGAEMTIHNGIIVPWICDTSPHNSESTSVFLPFVQQVRENRNRHIKGSLEEKFWKEIGNSLYGKLAQGLRAKTAFDTARGLNRSLPPSSVTQPFFAAHVTGFIRAVVGELMNALPSDSSVVSVTTDGFLTNCPLDKINMSGPLSSRFQSLCDIVDPGSSMLTCKHEVSQLIAMKTRGQLTYKAIQGKPVVHARAGVKPPADIPRSDYNDYMVDLYLNRLPGQTLSRSTLISTREMWLSESDLVSREQDIRLNLEFDFKRQPVRPAMNEGHLLMFSRPWDNMEEALQQRSLFDDWRQTHTLKTLADWDDWCDFLYCRTVFSDMKLKVGSKRSDDILVRLFLRALTQCQWGLMLKDKKSYSCKEVAEWLTSEGYSVTVTDVKNAVRAKIPQMKFSSVTPRMKSLMDIIARKYPTFCLPA

SEQ ID NO: 24 - protein, 866 aa, Escherichia coli
MSHNLQDILAAASGYQSVTSEPALNRKRPKTLDDYPVIPPASKKVSVISSDLTLHIGFDTEYVFNPETRQNDILSYQSYVVLPDNTGISNIIYPPDSQKKSRLSFKDFLCQTITPLLETGVITKWPGIINIYAHFIRADIASFANFWSDYKILLKGIRGTVSSFKNRYGIDFDEQQERRVKTEQIMFDKRTSPPRCSNVAFIDTLLITPGGMGLAECGELLGLPKLTIPAPYSITNMREYLLGDRAGFEAYALRDAEIAVRYALQVRNFCARELMIDRVPATIGAMAVSRFTKTLKENNMSPEVCLGTHIKTRELWLTEKQAFRTIKNPASVPSRELFETFPINCYHGGRNECFMMGVTPSDHWYDYDLAGAYTTGLLDILTPDYGNIRLSKNPDDYCGHVMGFALVTFRFPESVPYPSLPVRTDQYGLFFPLSGESWATAPEIELALSLGAEMTIHNGIIVPWICDTSPHNSESTSVFLPFVQQVRENRNRHIKGSLEEKFWKEIGNSLYGKLAQGLRAKTAFDTARGLNRSLPPSSVTQPFFAAHVTGFIRAVVGELMNALPSDSSVVSVTTDGFLTNCPLDKINMSGPLSSRFQSLCDIVDPGSSMLTCKHEVSQLIAMKTRGQLTYRAIQGKPVVHARAGVKPPADIPRSDYNDYMVDLYLNRLPGQTLSRSTLISTREMWLSESDLVYREQDIRLNLEFDFKRQPVQPAMNEGHLLMFSRPWDNMEEALQQRSLFDDWRQTHTLKTLADWDDWCDFLYCRTVFSDMKLKVGSKRSDDILVRLFLRALTQCQWGLMLKDKKSYSCKEVAEWLTSEGYSVTVTDVKNAVRAKIPQMKFSSVTPRMKSLMDIIARKYPTFCLPV

SEQ ID NO: 25 - protein, 903 aa, Enterobacter sp. MGH85
MNKKSNFLRIFAQPLSDFPSISGVDNDTAHLNKKKILMFDMNALLANAAGVTQSDSRPTKTRDNFPLIPQKSKKRLDVSSQLHLDIGFDTEYVYNPQTKQNDILSYQSYVVLPDGTGVPGILYPASAHKKDRLSLKNFLAKTLTPLLKNEQITEWPGSITLYAHFLRADVASFSDFWSDHKILLKGIRSTVSSFKNRYGIDFDEVENRREKNSLITFDKRTSPPRCSNVMFTDTLLITPGGMGLAECGQLLGLPKLTIPAPYSISDMRQYLKGDRRGFEAYAVRDAEIAVRYALQVKSFCTESLMIERIPTTIGAMAVSRFLKTIKESGQSPEVCMGTWTDSRQRWNPDTQGFRTLKSTQSIPARELYETFAINCYHGGRNECFMMGITPESQWYDYDLAGAYTTGLLDILQPDYDNIYQSQNPEEFCGHTMGFALVSFRFPDTVRYPCLPVRTDQYGLFFPLTGESWATAPEMALALSLGAEMTIQHGIIIPWRQYKSNDSSSPAEPVCSVFLPFVQQVRENRNRHDKGSLEEKFWKEIGNSLYGKLAQGLHAKTAFDTARGLNSPLPPSSVTQPFFAAHVTGFVRAVVGELMNALPPNATVVSVTTDGFLTDSAIENIDMSGPLSSRFQALCGIADPGSSMLTCKHQVRQLVAMKTRGQLTYKELAGYPIVHARAGVKPPADIPRDDYNRYMVDLYLNRAPGQKLRRGSLISTRDMWLNESDLVAVESDIRLNLEFDFKRQLIAPTMNDGHLLMYSRPWNDIAQALKQRQLFDDWRQTHSLKDEADWEDWCDFLYCRNIFTPLKLKVGQNRSDDVLVRLFLRALAQYQWGLTPDDRKRQTSVEIAAWLVEAGYSVTPSDVKNAGRAKLPPIIFDSLTARMNRLMDLIKLVYPGFALPSAVL

SEQ ID NO: 26 - protein, 866 aa, Enterobacter cloacae
MFDMNALLADAAGVTQPVARSAKTLDNFPLIPQKSKNRLDVSSELHLDIGFDTEYVYNPHTKQNDILSYQSYVVLPDGKGVPGILYPASAHKKDRLSLKNFLAKTLTPLLKNEQINEWPGSITLYAHFLRADVASFSDFWSDHKILLKGIRSTVSSFKNRYGIDFDEVENRREKNSLITFDKRTSPPRCSNVTFTDTLLITPGGMGLAECGQLLGLPKLTIPAPYSISDMRQYLKGDRRGFEAYAVRDAEIAVRYALQVKSFCTESLMIERVPTTIGAMAVSRFLKTIKESGQSPEVCMGTRTISQQCWNPDTHGFRTLKSTQSIPARELYETFAINCYHGGRNECFMMGITPESQWYDYDLAGAYTTGLLDVLQPDYDNLYTSQNPEEFCGHTMGFALVSFRFPDTVRYPCLPVRTDQYGLFFPLTGESWATAPEIALALSLGAEIAIQHGIIIPWRQYKSDNASSPTKPASSVFLPFVQQVRENRNRHDKGSLEEKFWKEIGNSLYGKLAQGLHAKTAFDTARGLNSPLPPSSVTQPFFAAHVTGFVRAVVGELMNALPPNATVVSVTTDGFLTDVSLENIDMSGPLSSRFQALCDIADPGSSMLTCKHQVRQLVAMKTRGQLTYKESEGFPIVHARAGVKPPADIPRDDYNRYMVVLYMNRAPGQKLRRGSLISTRDMWLNESDLVAVESEIRLNLEFDFKRQLITPTMNEGHLLMHSRPWDDMSQALKQRQLFDDWRQTHALKDEADWEDWCDFLYCRNVFTPLKLKVGQNRSDDVLVRLFLRALAQHQWGLTPDDRKRQTSVEIAAWLVEAGYSVTPSDVKNAGRAKLPPIIFDSLTARMNRLMDLIKLVYPGFALPSAVL

SEQ ID NO: 27 - protein, 962 aa, Aeromonas eucrenophila
MKRQEKPTDNAGGTAVSFPYADANLQPDLNNRPPHGGYDMFNDAQHQSALALAIESALDPCQYMNSPSHDPGWVMNGLSTDVIAGDPDIPDYLLPVQENSTDKALRLRTQHYLKPGETVVPAKGSVLHIGIDSEYVYNPKTKHNDILSYQFFVITEKGEHAEVIYPASSKKSDRLSFERSISHIVVVCKEKGLITEWPKHVFVYAHFLRADLASFGDFWLFKTQMDGIRKTVASINSAYGIDLDNILRRRAKPTPLILRDKQRKAQRTLLTFVDTMLHTPGGAGLAAVGELIDLPKLSLPAGHSIERMDELLAGDKAAFEAYALRDAEIAVKYGLRLHEFAKTLGLSSLPKTIGGCATSVFLKHLRETAQDRDQLFGTHEVEQTGWSKNSSRPVTKKVREMTPAAKLFENLAIDCYHGGRNECFWCGPTPLSLFNDFDLSGAYTTGLVDLFPLDYERARMTTNTAEFCGHVFGLARVKYRFPYGTRYPSLPVRTEIGLLFPLTGESLCTAPEIEVALRMGCQIEIHQGVIIPWTDTTQRLFEPFVSQVREKRQSYVKKSFEELLWKEIGNSLYGKLAQGLRGKSAFDTSSGLSKPIERSAITNAFFAAHTTGLIRAVLGEVLASIPAHRTVVSVTTDGFLTDATYDELVLNGPICRRFQELGERLDGPGFRMLEQKHQVKQVIAMKTRGQLTPEGVEGQPQILAKAGVKPPCSKELHQAYMLDLYLNRTPGQKVESDHLISTAEMWINEHDLVSVSRSKTLNLEFDFKRQPMLPSMQSVLGTEHICFDTRPWPTVAAAMEQRVVFDNWRRTNCLKTLNDWESWEDYFVCKTSIKGLPMRVTDEGSLGILKRVFLRAYTQSAFGMTKTMGYDELAEWLTINGCPTSVDDCKSAKRAKLVGQCVPVTTRTVRLVRVILQECPGLELGALFKPEDMPQLQSRLNNPKTEIAQITQDAPSHEVITD

SEQ ID NO: 28 - protein, 947 aa, Aeromonas hydrophila YL17
MSIHNQPPLQSGTAVAMDCPINDSLFAFPEPDAMTVNEDYAQPDISYEQLELARSIQLALDPSTYILDSRNAVDPIMRGQSASAEEDLLLKKALTRLRAGETVTLAKGEPIHIGIDSEYVYDPKTKRNVILSYQFHVITELGSHSGIIYPKSGKVSDRLEFDPFIARIVIMCKEKGIITKWPKKIYVYAHFLRADLASFSDFFRKKTKVSGIRKTVTTMTETYGVDIKALLARRAQPEPMILKDSQRKKHMTLIAFVDTMLHTPGGTGLATVGEMIGIPKLSIPDGYSIERMDELLAGDKSAFEAYALRDAEIAVKYGLRLHEFIKQHGLTRLPASLGSLSCSMFLKFLRDQEYDQHQLLGTEVVERSRWNDKESRLTSQKLRQMTSLARTFEPLAIDCYHGGRNESYWNGPTPVSSFYDFDLSGAYTTALVDLFPLDYGNARLTSNPEDYRGHVLGLARVRFSFPTGLRFPCLPVFDEKYGLLYPLSGESNCTAPEIEVALNMGCQIDIIQGIIIPWCDVEVSPFESFVSFVRKMRKSYTKKSCDELLWKEIGNSVYGKLAQGLQGKTAFDTTTGLSKKIDRSAITNAYFAAHTTGIVRAVLSEILAAIPANKTVISATTDGLLTDATYEELDLSGPLCRRFQALGERLDGDSFRMLELKHGANQLIAMKTRGQLTAIPMEGQPDILAKAGVKPPCSKDQHQNYMLDLYLNRTPGQKVDSEQLVSISEMWINECDLVSMTKTKTLNLEFDFKRKPMQPSMQSVLGIEHICFETQPWPTAQAAIEERIIFDSWRKNHCLKTLEDWENWEDYLTCKGSMKSNVMRMTDEGSLGILKRVFLRAYTQSAFGMTKTMGYSELAEWLTVNGCPTSVDDCKSAKRAKLVEQCVPVTTRTVRLVRVIMQECPGLDLGALFKPEDMQQLQGRLNNPKTEMAQITQDAPSHEVITD

SEQ ID NO: 29 - protein, 627 aa, Photobacterium kishitanii
MSEVKFFNNMVAIDGEADLSAFMHDMASPPIIPDTQMSNDIPVDIKSGLMALENDIPSEPFPIGLPAYQLMTLEWASGETLYAGFDTEYQHNAITGQNEIISYQVVGQTQRGQCSVIVYPKSGAKHHRWTFEALVGHVLEQMFEQELLDEVPKQVVVFGHFLRADLTTFSDFWKKQKTTLRGVSRTVTSAMQDYGVDVHALCKRKAGKDPHVVEAPSGEKYRTKVRFVDTLALSPNGSGLAVIGRLIGLPKLELPDGYAKDEMRRFKDEKPDLFYSYAMRDAEIALAYGLRMFKFATVELGLSKCPITLGAMGVAVFQKMLKETGVDKRDVFGEREITTQHWNAKLGRPHTKKELVPTDARELFEHLAIRCYMGGRNESFTCGPSDIGTFYDFDLVGAYLGGMVDIYPLDYDRAYMSIDVNAFCGHVCGFARVRFSFPDGTRFPCIAVHHDLYGLYFPMTGETYTTAPEIEAARNMGATIEILQGVVTPWQHDSELLFLSFVQLIREKRTSYPKKSYEESMWKEIGNSLYGKTAQGLRTKTAFELVSGLNKDIPRSAVTNPYFAAHTTGFIRAVIGELLASVPTNRQVISVTTDGFLTDAPMNELDLTGPLCARFNAHNELVTNYLN

SEQ ID NO: 30 - protein, 623 aa, Vibrio ponticus
MSENPQFFNNLVAIDEPDVSLFLGNDLGLPDLSGMSFSNDVPDDVKPELMTLANDIPTEVMGYEPMSLEWASGETLYVGFDTEYQHNAITGQNEIISYQVVGQTQRGQCSVIVYPKSGAKHHRWTFEALVGHLIAAMFEQEQLDEVPKQVVVFGHFLRADLTTFSDFWKNQKTTLRGIRRTVTSAMQDYGVDVHALGKRKAGKDPHVVEAPSGEKYRTQVRFVDTLALSPGGSGLAVIGELIGLPKLDLPDGYAKDEMRRFKDEQPDAFEAYAMRDAEIALAYGLRMFKFSTVELGLSKCPTTLGAIGVSVFQKTLNESGVDKRDAFGEREITTQHWNAKLGRPHTKKEFIPTEARELFERLAIKSYFGGRNECFTCGVTEVGTYYDFDLSGAYTTGMVDLRPLDYENAFMSRSMNDFCGHVCGFARVRFSFPNGTRFPCLPVHHELYGLYFPLTGETYATAPELEVARNMGAHVEILQGVVIPWMVESEPLFLPFVRLIREKRTSYPKKSFEEATWKEIGNSLYGKTAQGLRDKTAFELANGLTKDIPRSAVTNPYFAAHTTGFVRAVIGELLASIPEHRQVISVTTDGFLTDATKEELNLSGAMCLRFNEHDQMIMTTNFK

SEQ ID NO: 31 - protein, 593 aa, Aeromonas media
MFEFKKAEIGVIEEDQPEPPHLKFAIKKVSFDPKQPPISFADGEDLWIGVDAEWVTRDGQNIVLSYQVYCVNSRDETLGKVIYPELGKRLAFETLISMAVEDCRAAGLIKKWPRKIVVVAHFLRADLSTFKDFWSMKTRLDGQGGSVVGQIITDSGYGVDETAERKRRAPLKPITLRDRNRKLRKSIIQFVDTLFLSPNKSPLSALGSMLGLPKVEIPEGYSIERMDELLVGDKEAFERYALRDAEIAVKYALKVRDFLGGQFGLQKLPRSLGAVGVAVFRQLLKAADVDYMAAFGLVIKKEERWNSGKGKVATKAVKRPSPDRWRCEALAICCYYGGRNESFMIGPTPIGDWYDWDLKGAYTTGLCDLLEPDYANMYTSSDPQDFIGHVMGFAYVEFAFPAGTRFPCLPVRSEQYGLRFPLSGLAYVTAPEIELALSMGATIAIKHGVIVPWVAGSQPLFEDFTRMIQRLRREYPKKSLEEVMVKEIGNSLYGKLAQGLSDKTAFDTATGLSKKIGPSAVTNPYMAAHTTGLIRAVCGELLHRIPSHRTVVSVTTDGFLTDAPLEELDQTGPLCRRYQALCQRLHGDEEVGQ

SEQ ID NO: 32 - protein, 896 aa, Aeromonas allosaccharophila
MWLVPALYYGRLEIMGDHVVLVWRNLMFEFKKAEIGIIEEDQPAPSHLPFAIKKATFDPKQPPISLADGEDLWVGIDAEWVTRDGQNIVLSYQGYCVNSRDETLGKVIYPEPGKRLAFETLISMAVEDCRAAGLIKKWPKKIVVVAHFLRADLSTFKDFWHMKASLDGQGGSVVGQIITDSDYGVDETAERKRRAPLKPITLRDRNRKPQKSIIQFVDTLFLSPNKSPLSALGSMLGLPKVEIPEGYSIERMDELLVGDKEAFERYALRDAEIAVQYALKVRGFLGSQFGLQKLPRSLGAVGVSVFRRLLKDADIDYMVAFGLELAKIERWNTGKGKVTTKAVTRPSPARGLYEDLAIRSYHGGRNESFMIGPTEIGDWYDWDLKGAYTTGLCDLLVPDYANMHTSSDPQDFVGHVMGFAYIEFTFPAGTSFPCFPVRSEQYGLRFPLSGLAYVTAPEIELALSMGASIHIKHGVIVPWLSGSGPLFEEFTRMIQRLRQEYPKKSLEEVMVKEIGNSLYGKLAQGLRDKTAFDTATGKNNKIGPSAVTNPYMAAHTTGLIRAVCGELLHRIPLHRTVVSVTTDGFLTDAPLEELDQTGPLCRRYQALCQQLHGDESGDPVPMLELKHHARQIVSIKTRGQCTAIQGDTPPVLAKAGVKCAGTTEEQNEWIMRLYLDREPGQKIDASHLISLREQWLTESDLIEIKKQSRLSYEFDQKRQLVNPQIVEVAGGSHIACDTVPWGDAGMADHCRARFEGWREDNCLKTLEDWASWEDYYESALALQGSKMRVREDGSLGILTRILTRSLVQKAWFDHTMTYGEISALLTSVGLPVTVDTCKNSKRAALPENVVPVTGEVLRVLALLLRQVPEYPLEPLFKPERLDEVKSRLNSMEISHA

SEQ ID NO: 33 - protein, 912 aa, Aeromonas allosaccharophila
MKSEHKMPLERVPLPYTPSFLAESITQLFMLDPPDLRELMTPPPSGDAAPDLTDLFTPPNPFALMKTPGSATRPLDLAPVTLADGADLYVGLDAEWVADGNRNQVLSYQTYCINEDGTELGKIYYPDAGKRFGFEDLISMMVEDCRAAGVIKEWPRKIIVVAHFLRADLSTFQSFWKMKTRVNGQGGSVVGRVLTDSGYGVDETTVRSRKASPAPILLKDKHRKPQKSIIQFVDTLFLAPNKSPLSALGDMLGLPKVEIPAGYSIERMNELLAGDKVAYERYALRDAELAVKYALKVQDYLAHEFKLTALPRSLGAVGVNVFRRLLAEHGIDDMASFGMRSVSHVEWNARNGKVTTKRNKRSNPSRCLFETLAIDCYMGGRNESFMVGPTIEGHWYDWDLKGAYTTGLCDLLVPDYAKAYMTDNPNAFVGHVMGFAYVTFKFPAVTRYPCIPVRSEQYGLRFPLEGDAYVTAPEIELALAMGATIEIKHGVIVPWVVNSPRLFESFTSMIQKRRKALPKKSLEEVMIKEIGNSLYGKLAQGLSDKTAFDTATGLSKKIGSSAVTNPYMAAHTTGLIRAVCGELLHRIPLHRTVVSVTTDGFLTDAPLEELDQTGPLCRRYQALCQQLHGDESGDPVPMLELKHHARQIVSIKTRGQCTAIQGDTPPVLAKAGVKCAGTTEEQNEWIMRLYLDREPGQKIDASHLISLREQWLTESDLIEIQKKIRLSYEFDQKRQLVNPRMVEVAGETHIACDTVPWDDAGMADHCRARFDGWREDNCLKTLEDWASWEDYYESALALQGSTMRIREDGSLGILTRILTRSLVQKSWYDHTMTYGEISALLTSVGLPVTVDTCKNSKRAALPENVVPVTGEVLRVLALLLRQVPEYPLEPLFKPERLDEVKSRLNSMEISHA

SEQ ID NO: 34 - protein, 905 aa, Ferrimonas senticii
DRQIKIFFDGVRSAPWAALRGKGKAVHIAIDSEWVFNPETGKNDILCYSYCVRAGDKTFKGVKSTEMAKLIKQCRDQGLTKDEEMLKRKQLANSTKGYKANFDQFIQELLLKAKARGFIDEWPEHTFIYAHFLRADIASFDEFWNIGTKGKNKANCFTAVQGSITSGRGAYGIDLASIGRSKYKTENTKFYCGGNNVIETKVRFIDTMLLSSKASLDDIGELVGIPKMNLADGMIARMDDLYCEDRGLFERYAVRDAQIALEYGLKMQQFALVDMREDTGLELKQLPSTLGNFAVSLFKHTGGGVDQMHEFLGYEKRKSEYFHAKSNGIRKSVTIAKTVSREYTDALAVHCFYGGANFGAYFGVTEQGDYNDYDLSGAYTTALVDILEADYLNSFESKNLEDYLGHTMGFAYVRFKHPEGTKWGLLPCRTDLRGIYYPLEGETYVTAPELQLAHDAGVEIEILHGQVIPWKSGSVSQFKAFTKIIREQRSKYKREGNELYDQLWKLIGNTLYGKVGQGLREKSGFDVSSGLSSKIPYSPVTNAHYAAHATGFVRATMMEIIRKLTMDEQVQIVSATTDGFLTNATQEQLDKCLDGPLAKRFQHICNEVSGEDMMQLKHHAKQIVSMKTRGQLTTELGDTKPVCAKAGVKPPKGVDENAWMVELFLDRYPKQKIERSHLASAREMWLKELDLISIHTEQTLNLEWDFKRRPVTPRMVTVRHPVSGEIVEHLSFDTVPWSTVDEALDARTYFDEWRASHCLKTMEDWESWMDFYKVRRYLKGTGVKYLEDGSEGIFKVQMLRAIVQGGWGLPEAPQRAPRGHYDKLVAMFDVDGIGGITKQDLANAKSRKLLTARLPITSRMLPLLSWFARQYPTVDLTLVFHPDEVDDAVLMLETYNADAAEKLAA

SEQ ID NO: 35 - protein, 964 aa, Vibrio vulnificus
MNIFEQEAKANYQLMRQTDREVGDFLVNTFSNNRSYILDDQVAKFQQELRTREEVKKTVDEQVKRYFEGLRSAPWAAIRGKGKAVHIAIDSEWVFNPETGKNDILCYSYYVQVGDKFFKGVKHTEMAKLIKECRDQGLSKEEEMLKRKQLANSTKGYKVNFDKFIQELLIKAKSRGFIDEWPEHTFIYAHFLRADIASFEEFWNIGAKSKNHKNSFTAVQGSITSGRGSYGIDLASIGRSKYKTENTKFYTGSNNTFETKVRFIDTLLLSSKASLDDIGELVGIPKMTLADGMISRMDDLYCEDQSLFDRYAVRDAEIALKYGLQMQRFALVDMREDTGLELKQLPSTLGNFAVSLFKHTCGGVNEMHEFLGYEKRKGEYYHAKSNGTRKSVTIAKTVSREYTDALAVSAFYGGANFGAYFGVTEQGDYNDYDLSGAYTTALVDILEADYLNSFESKNIEDYLGHTMGFAYVRFKHPEGTQWGLLPCRTDLRGIYYPLEGATYVTAPELQLAHDAGVEIEILHGQVIPWKQGSVSQFKAFTKIIRKQRSKYKKEGNELYDQLWKLIGNTLYGKVGQGLREKSGFDVSSGLSSKIPYSPVTNAHYAAHATGFVRATMMEIIRKLTMDNDVQIVSATTDGFLTNATPEQLESCLDGPLAKRFQRICKEVSGEDMMQLKHHAKQIISMKTRGQLTTELGSTKPVCAKAGVKPPKGVNENAWMVELFLDRYPKQKIERSHLASARDMWLKEMDLVSIHTEQTLNLEWDFKRCPINPRMVKARHHVSGEMVEHLSFDTVPWNTVDEGLDARTYFDEWRVNNCLKTMEDWDNWMDFYKVRRYLKGTGVKYLEDGSEGVFKVQMLRAITQGGWGLPAVPQRAPRGHYDKLVAMFDADGIEGITKQDLANSKGRKLLESALPITTRMLPLLSWFARKYPTVDLTLVFHPDEVDEAVLMLEEYNLKCTEKLVA

SEQ ID NO: 36 - protein, 965 aa, Vibrio tasmaniensis
MKTLETTPKTTYQLMRETEHELEDFLQSTFFDTKSLLLDDQVSKFEAELRGREEAKKEIDKRINRYLEGIKSAPWAAMRGKGKAIHISIDSEWVFNHETGKNDILCYSYSVRIGDKSFSGVKHTDMAKLIKQCRDQGLSKEDEMDKRKQLTKKGYKIGFDKFIQELLIKAKARGFIEEWPEQTFIYAHFLRADIASFEEFWNIGKNNKNHKNSLTVVQGTVTSGRGAYGIALDSIGRSKYKIENTKFNSSSNNAFETKLRFIDTTLLSSKASLEELGLQCGFPKMTLPDNMIERMDDLYCKDTSLFNRYAVRDADIALEYGLRMQKFALVDLREDIGLELNSLPSTLGNLGVSLFRHTCGSTAAMHDFLGYETRKKQYYHAKSNAIRNTYDISKTVSREYTDNLAVSALFGGCNFGAYFGVSEKGDYFDYDLSGAYTTSLVNSKKADYPNTFESKNIEDYLGDTMGFAYVRFKHPDGILFPVMPCRTDLRGIYYPMEGETYVTSPELQLAHDIGCEIEILHGMVIPWVEGSTSMYKDFTTIIRKQRSKYKKEGNELYSGLWKLVGNSLYGKTLQGTSSHTKGFDLATGLSKNIPYSPVTNAHYGAYCTSYVRATMLEVIGKLCERYGDDIKIISATTDGWLCNATQEQLEQCLDGPLARRFQQICTEVSGEDMMQLKHHAKQIISMKTRGQLTAELGDTKPVCAKAGVKAPKGVDENEWMVELFLDRYPGQKVARKHLVSARDQWLKELDLISIHTEQTLNLEYDFKRRPVNPRMVEVRHPKSGEMIEHLSFDTVPWNTVDEGLDARTYFDEWRVNNCLKTMEDWDNWMDFYKVRSYLKGTGVKYLEDGSEGIFKVQMLRSITQGKWGLPEDPKRAPRGHYDKMVATFEADGIEGITKQDLANSKGRKLLESKLPVTPRMLPLLSWLVRKYPMADMTLIFHPIEVEEAVSMLEEYNREHTEKLAA

SEQ ID NO: 37 - protein, 960 aa, Vibrio campbellii
MNIFEQEAKTNYQLMRQTDREVEDFLVNTFSNNRSYILDDQVAKFQEELCSREGAKKTVDEQVKRYLEGLRSAPWAAMRGKGKAVHIAIDSEWVFNPETGKNDILCYSYCVQVGDKSFSGVKHTDMAKLIKQCRDQGLSKDEEMDKRKQLTKKGYKISFDKFIQELLIKAKSRGFIDEWPEYTYIYAHFLRADIASFEEFWNIGINNKNRKNALTTVQGTVTSGRGAYGIDLDSIGRSKYKIENTKFYSSSNNAFETKVRFIDTMLLSSKASLEELGLQCGFPKMKLPDNMIERMDDLYCNDISLFNRYAIRDAAIALEYGLRMQKFALVDLREDIGLELNSLPSTLGNLGVSLFRHTCGSTAAMHDFLGYETRKKQYYHAKSNSIRNSYDIAKTVSREYTDNLAVSALYGGCNFGAYFGVSEKGDSFDFDLSGAYTTSLVSCLKCDYANTFESKNIEDYLGHTMGFAYVRFKHPEGIRFPVMPCRTDLRGIYYPMEGETYVTSPELQLAYDIGCEIEILHGMVIPWVEGSTSMYKDFTTIIRKQRAKYKKEGNEMNSHLWKLIGNTLYGKTLQGCNNSKGFDLATGLSKNIPYSPVTNAHYGAYCTSFVRATMLEVILRLPSEVQLISATTDGFLTDATPEQLEQCLDGPLAQRFQQICNEVSGEDMMQLKHHAKQIISMKTRGQLTAELGDTKPICAKAGIKAPKGVDENEWMVELFLDRYPGQKVERKHLASARDQWLKELDLISIHTEQTLNLEYDFKRCPINPRMVKVRHPVSCEMVEHLSFDTIPWNTVDEGLDARTYFDEWRVNNCLKTMEDWDNWMDFYKVRRYLKGTGVKYLEDGSEGIFKVQMLRAITQGGWGLAAVPQRAPRGHYDKLVAMFDTDGIEGITKQDLANSKGRRLLESALPMTTRMLPLLSWFVRKYPIVDLTLVFHPDEVDEAVMMLEEYNLKCTEKLVA

SEQ ID NO: 38 - protein, 964 aa, Vibrio parahaemolyticus
MKTLETAPKTAYQLMRETERELEDFFQSTFFDTKSLLLDDQVSKFEAEMRGCEEAKKEIDERINQYLEGIKSAPWEAIRGEGKAIHISIDSEWVFNQETEKNDILCYSYSVRIGDKSFSGVKHTDMAKLIKQCRDQGLSKDEEMDKRKELTKKGYKKSFDKFIQELLIKAKARGFIDEWPEHTFIYAHFLRADIASFEEFWKIGTSNKNHKNSLTVVQGTVTSGRGAYGIDLDSIGRSKYKMENTKFYSSSNNAFETKLRFIDTTLLSSKASLEELGLQCGFPKMTLPDNMIERMDDMYCKDTSLFNRYAIRDADIALEYGLRMQKFALVDLRKDIGLELNSLPSTLGNLGVSLFRDSCGGAAEMHQFLGYEKRKNQYYHAKSNSIRNSVELAKTVSREYTDALAVSAFYGGANFGAYFGPTEVGDYNDFDLSGAYTTALVDILEADYLNSFESKDIEDYLGHKMGFAYVRFKHDDKENFGLLPCRTSLRGIYYPLEGETYVTAPELQLAHDAGVEIEILHGQVIPWKNGSTSKFKEFTKTIRKQRAKYKEKGNELYEKLWKLIGNTLYGKVGQGLRDKSGFDLASGLSSKIPYSPVTNAHYAAHATGFVRGTMLEVMRKLNERYGDDIKIISATTDGWLCNATQEQLEQCLDGPLARRFQQICTEVSGEDMMQLKHHAKQIISMKTRGQLTAELGDTKPVCAKAGIKAPKGVDENEWMVELFLDRYPGQKVARKHLASARDQWLKELDLISIHTEQTLNLEYDFKRRPVNPRMVEVRHPKSGEMVEHLSFDTVPWNTVDEGLDARTYFDEWRVNNCLKTMEDWDNWMDFYKVRSYLKGTGVKYLEDGSEGIFKVQMLRAITQGKWGLPEAPKRAPRGHYDKMVAMFEGDGIEGITKQDLANAKGRKLLESALPITSRMLPLLSWFVREYPMVDMSLIFHPDEVDEAVLMLEEYNLDHTEKLAA

SEQ ID NO: 39 - protein, 951 aa, Vibrio vulnificus 93U204
MKNDASKDQQKALEQEVEVFLQQESSDHSTTETEEGLTDFLEMESQSHYSSKAVEEELDIFFENENQPPWKALKGDDESVHIGIDSEYVYNEEENRNDILSYQYYLIAGKNEISDVILTPVAEVIKKSRAANKSREDELKAINKVKKPRKKFEEFLVEILQEAKNRGFIKGWPRTIYIYAHFIRADLVSFDAFWDTSQKAKLEVIRGTIASTRGSYGIDLNAVGRTKQATEPVHFTDKHGKKRESRVRFVDTMLLSPGQSGLDSAGELIGIKKEVIPTPYRKDRMDELLVADEVRFLRYALRDAEITVKYGLEMQRFALEDIRKALKTKLPKAQLDKLQFKHLPSTLGNFSVSVFKALTGDKEALNEALGMETKETHYWNHLQKRVSTRKDTVITAGRRIFEQLAIDSFHGGRNECYVFGGGVVGDYNDFDLATAYVNALMDINPVEFEKSFTSTNVKDYLGHKMGFAYVKFTFPSETRFPCLPVRTDIYGLYYPLEGYSYCTAPEIEVAKNMGCKLEIQFGVVVPWKEEEESLFKGFTELIREQRQKYTENNDKFREKLWKEIGNTLYGKLGQGLRGNRGFNASTGLSKDIPHSPVTNPYFAAHATGFVRAVLSEQIAGLPDTIDVISATTDGYLTNATEAQLYTSGSVSQRFAAICQQTGDGKMIKHKHHVRQVIAMKTRGQLTGEHGKSEPVIAKAGVKPPESTLSSKKDENAYMVKLFLDRYPGQKIPNNSLISPRDMYLKDMDLIEIQREKVLNLEFDFKRKPVNPRMTQIRHPDGHIVEHLYFDTVPWKNALEGQRVRAMFDGWRKSNCLKTMEDWENWIDYAKTKPLLKGSHIKYDESGSYGVLLKLAVRALSKESYGLTKTINGKKLTLKQLTDLFNNAGFEIAENAIGNSRDTVFRPNVLAATPRLMPLLSWLVTVFPEMELEAFFHEDELDEAKKMLKAFR

SEQ ID NO: 40 - protein, 1004 aa, Vibrio splendidus 12B01
MTKSLSSSDNAEKEYVSTTSFSPILGAQATERATTSAQLQDFIDTWRYRFEPEYQRDSTLELGEYLKSRKQPIKEEGVVAKELTAHLSARKSRFKYLQAQGGNVHIGIDTEFEYDEENECNLILSYQYCLLTADGREFKGVDYPKSTKKEDRFDFNDYIFKIINRAKKHGWISEYPEKTFIYAHFMRADLASFHAYWNIKSNKLDAAKDAVNSARGDYGLDLRAIGASQYKPRFVSYKDNSKRTVKTTLHLKDTLFLSPGRCSLDVIGDAIGIPKIKIPDGYSIEKMSKLLKEDKGAFEQYAIRDAEIAVKYGRYVEDFALTELNDVFEDEGSDDQRPASNRIKYLPNTLGNLSVSLFKNVFADDYAKKVQVNDDSVLPASASLNNIFGMEEVISYKWDERNHRSIPNKLLVLSGERDRNEATARRCFFGGRNEDYYFGPSPVGKVSDWDLAGAYTTGLVDILPVNYRAAFSSTKIEDYLGHVMGFAYVKFKFKAGTRFPSLPVRTEVYGLYYPLEGETYCTAPEIAVAYNMGCEIEILYGDIIPWADDAEPVFEPFTKVIRKLRKRHKGTFEEKIVKDVGNTLYGKIASGVGFQRNKFDTKTGLSKASGTSPVTNSYFSSHVTGFIRGVLSELLANVDEGVTVYSATTDGLLTDLDNADSMLVDEYHLKGKTYQSTTARFKALCAKFGDDEALVLKHQVKQIIAMKTRGQLTAEMMVDDGTNPDMSGLYKKPVTAKAGIKPPRDCPNENDWMVNLFLNRQPSEKIANNCIVSERDMYLHELDLIEIKHDKYLNLDFDFKRRPVNPSMVVVRNPVTGEVVSHLTFDTVPWQTHIEGEKARSAFDGWRKGQLVGKKPNQERVGGNCLKTMDDWRNWMDFYKIKAVMEVKGQKYEDDSSDGIFKRYVMTAITNDLWGMTKETVEGVKRTYPDLAGLFTRAGYSTIGKDFSNAKGRQVVANMMPAAPKLIPMLIWLMGEFPDMEVDKFFIPEELDEVMTLVASARDK

SEQ ID NO: 41 - protein, 1051 aa, Moritella viscosa
MTTTLSPEQTKDEQDEKTVVSTPVKKSDKYVSTISYSTIRGGEATERATQDAQLQNLMDGIRRRFGPEYQKDSTTELRKYLANRVKPIKENKDVEKELIHYHIDRKSRFKYLKAQGSNIHIGIDTEFEYDEENECNKILSYQYCLLTADGREFKGVDYPASTDKKDRFDFNNYIFQIINYAKRHGWLSEYPEKTFIYAHFMRADIASFDAYWNIKSNKLDAVKAVASNARGDYGLDLRAIGASQYKPKYVTYKNNGKRLERTTLHLKDTLFLSPGRCSLDVIGEAIGIPKIKLPAGYSIEKMSKLLEENKGAFEKYAVRDAEIAVKYGRYVEEFALTELNDVFDNDDSEANDAGAVSEGGAKTKNSSSNRIKYLPNTLGNLSVALFKNVFADKYEKRAAEAESYTAPLIPNMAFNEVFGMEEVISYKWDERRHRSIPNKLTVLSGERDRNESTARRCFFGGRNEDYVFGPSAKDAVSDWDLAGAYTTGLVDILPVNYRAAFSSTDIEDYLGHVMGFAYVKFKFDEGTRFPSLPVRTELYGLYYPLEGETYCTAPEIAVAYNMGCKIEILYGDIIPWVNDAEPIFEPFTKVIRKLRKKHKGTFEEKIVKDVGNTAYGKIGQGVGFQRNKFDTKTGLSKPNGNSPLTNSYFASHVTGFIRAVLSELLDNVDDDITVYSATTDGLLTDLGNADAMIIDEYDLDGKIYQSTTARFKALCARFGDDDALVLKHQVKQIIAMKTRGQLTAEMMEDDGTNPEMSALYKKPVTAKAGIKPPRDCPNENDWMVDLFLNRQPSEKVANNCIVSERDMYLHELDLIEIKHDKYLNLDFDFKRRPVNPSMVDVRNPLTGKTVSHLTFDTVPWKNHKEGELARSAFDGWRKGKLTPVEPSEEPSDETDKKSSKKPEKKPKKVRVGGNCLKTLDDWDNWMDFYKIKAVMTVKGQKYENDSSEGIFKRLVLTALTNDSWGLSKDTPDGTNRTYPELIKLFTNAGYPVKKSDFTNAKNRKIEEHMMPAAPKSIPLLKWVMSQYPDMEVDKFFMKEEFDEVMGLVNKS

SEQ ID NO: 42 - protein, 998 aa, Vibrio parahaemolyticus
MTTETAEATEIIENTKPAETTDTLSFSPILGVQATKRATDTAQLHNLIESWQKRFDLGEQQDKSLELQTYLENRKLPPKSFQALKSELAQYLKDRKSRFKFLKAKGGNIHIGIDTEFEYDEEAECNKILSYQYCLLTPDGKEYKGIDYPASAKKEDRFEFNDYLFKIIVRARKMGWITEYPENTFVYCHFMRADLASFHAYWNIKGSKKYDAAMATVNNARGDYGLDLRAIGASQYKPRAITYTNHNKRPEITSIHLKDTLFLSPGRCALSVIGDAIGIEKVELPDGYSIERMSQLLEEDKGSFEKYAITDAKITVKFGRFMEDVVLEELNSITGIASSGDGKRATNQIKYLPNTLGNLSVALFKNVSSDVYEQRKESKQTPNLTLNEVFGLEEVTAYKWDESSNRSIPYKLVVLSGERDRNEATARRCFFGGRNEDYYFGPSPKGEISDWDLVGAYTTGLCDIKPVDYRKAYSSTNIEDYLGHVMGFAYVRFRFKEGTRFPSLPVRTELYGLYYPLEGETYCTAPEIAVAYNMGCELEILYGDIIPWIDDAEPVFEPFTKVIRELRKKHKGTFLEAVYKDVGNTLYGKVGQNVGFQRNKFDTKSGLSRPATNSPVTNSYFSSHVTGFIRGVLSELLANVGDDKRVYSATTDGLLTDLSDGEAMLIDEYHLNGQSYQSVTARFKALCEKFGDESMLALKHQVGQIIGMKTRGQLTAEILDADINTPELNKIRKKVITAKAGVKPPRDCEDENAWMVDLFLNRKPSQRISNNCLVPERDMYLHELDLYEIKRDRFMNLEFDFKRRPVNPTMVDVRDPKTGCIVSHLAFDTVPWKNREEGEMARATFDGWRKGKKSGDSRVGANCLKTMEDWYNWIDFYKIKAVMKVKGQNYENNSSEGIFKRYILTAITNEFGGLSRVNRQGKRRTNAELAELFTSAGYPTNEKDVSNAKGRKLHSQMLPAAPKFMPMLRWAMTQFPDLELKMFFMPEELGEVLALLDQ

SEQ ID NO: 43 - protein, 853 aa, Enterobacter cloacae
MTQPVARSAKTRDNFPLIPQKSKKRLDVSSQLHLDIGFDTEYVYNPATKQNDILSYQSYVVLPDGTGVPGILYPASAHKKDRLSLKNFLAKTLTPLLKNEQINEWPGSITLYAHFLRADVASFSDFWSDHKILLKGIRSTVSSFKNRYGIDFDEVETRREKNSLITFDKRTSPPRCSNVTFTDTLLITPGGMGLAECGQLLGLPKLNIPAPYSISDMRQYLKGDRRGFEAYAVRDAEIAVRYALQVKSFCTESLMIERVPTTIGAMAVSRFLKTIKESGQSPEVCMGTRTISQQCWNPDTHGFRTLKSTQSIPARELYETFAINCYHGGRNECFMMGITPESQWYDYDLAGAYTTGLLDVLQPDYDNLYTSQNPEEFCGHTMGFALVSFRFPDTVRYPCLPVRTDQYGLFFPLTGESWATAPEIALALSLGAEIAIQHGIIIPWLQYKSDNASSPTKPASSVFLPFVQQVRENRNRHDKGSLEEKFWKEIGNSLYGKLAQGLHAKTAFDTARGLNSPLPPSSVTQPFFAAHVTGFVRAVVGELMNTLPPNTTVVSVTTDGFLTDVSLENIDMSGPLSSRFQALCDIADPGSSMLTCKHQVRQLVAMKTRGQLTYKELAGYPIVHARAGVKPPADIPRDDYNRYMVDLYLNRAPGQKLRRGSLISTRDMWLNESDLVAVESDIRLNLEFDFKRQLIAPTMNDGHLLMYSRPWNDIAQALKQRQLFDDWRQTHTLKDESDWEDWCDFLYCRNIFTPLKLKVGQNRSDDVLVRLFLRALAQYQWGLTPDDRKRQTSVEIAAWLVEAGYSVTPSDVKNAGRAKLPPIIFDSLTARMNRLMDLIKLVYPGFALPSAVL

SEQ ID NO: 44 - protein, 866 aa, Enterobacter cloacae; identical to SEQ ID NO: 26

SEQ ID NO: 45 - DNA, 2610 bp, Artificial Sequence
  Codon-optimized sequence encoding SEQ ID NO: 2
catatgagcaataacctgcaagacatcctggctgccgcttctggctaccaaagtgtcacctcggaaccggccctgaatcgcaaacgcccgaaaaccctggatgactatccggttattccgccggcgagcaagaaagtgagcgtgattagctctgatctgaccctgcatatcggttttgacacggaatacgtgttcaacccggaaacccgccagaatgacatcctgtcgtatcaaagctacgtggttctgccggataacacgggcatttccaatattatctatccgccggactcacagaaaaaatctcgtctgagtttcaaagatttcctgtgccaaaccattacgccgctgctggaaaccggtgttatcacgaaatggccgggcattatcaacatttacgcccactttattcgcgcggacatcgcctcgtttgcaaacttctggagcgattacaaaatcctgctgaaaggcatccgtggtaccgttagttcctttaaaaaccgctacggtatcgatttcgacgaacagcaagaacgtcgcgtcaaaaccgaacagattatgtttgataaacgtacgtctccgccgcgctgcagtaatgtggccttcattgataccctgctgatcacgccgggcggtatgggtctggcagaatgtggcgaactgctgggtctgccgaaactgaccattccggctccgtatagcatcacgaacatgcgcgaatacctgctgggtgaccgtgcaggttttgaagcgtatgcgctgcgtgatgctgaaatcgcggttcgctacgctctgcaggtccgtaatttctgcgcgcgcgaactgatgattgatcgtgtgccggcaaccattggtgccatggccgtttctcgtttcaccaaaacgctgaaagaaaacaacatgagtccggaagtgtgcctgggcacccatatcaaaacgcgtgaactgtggctgaccgaaaaacaggcctttcgcacgattaaaaacccggcatccgttccgtcacgtgaactgtttgaaaccttcccgattaactgctatcatggcggtcgcaatgaatgtttcatgatgggtgtgaccccgtcagatcactggtatgattacgacctggcaggcgcttataccacgggtctgctggatattctgaccccggactacggcaacatccgtctgagcaaaaatccggatgactattgcggccatgtgatgggttttgcgctggttacctttcgcttcccggaatccgtcccgtatccgtcactgccggtgcgtacggatcagtacggtctgtttttcccgctgagcggtgaaagctgggccaccgccccggaaattgaactggccctgtccctgggtgcagaaatgacgatccataacggcattatcgtgccgtggatttgtgataccagcccgcacaatagtgaatccacgtcagtttttctgccgtttgtgcagcaagttcgcgaaaaccgtaatcgccatatcaaaggttccctggaagaaaaattctggaaagaaatcggcaactcactgtatggtaaactggctcagggcctgcgtgccaaaaccgcattcgataccgcgcgtggcctgaatcgcagcctgccgccgtcatcggtcacccaaccgtttttcgcggcccacgtgacgggttttattcgcgctgtcgtgggcgaactgatgaatgcgctgccgtctgatagctctgttgtcagtgtgaccacggacggctttctgaccaactgtccgctggataaaatcaatatgtcgggtccgctgagttcccgcttccagagcctgtgcgatattgttgacccgggttcatcgatgctgacctgtaaacatgaagtctctcaactgatcgccatgaaaacccgtggtcagctgacgtataaagcaattcaaggcaaaccggtggttcatgcacgcgctggtgtcaaaccgccggccgacattccgcgtagtgattataacgactacatggtggatctgtacctgaatcgtctgccgggtcagaccctgtcgcgtagcaccctgatctcgacgcgcgaaatgtggctgtctgaaagtgatctggttagccgtgaacaggacattcgcctgaacctggaatttgatttcaaacgtcaaccggtgcgcccggcgatgaacgaaggccatctgctgatgttttctcgtccgtgggataatatggaagaagccctgcagcaacgtagtctgttcgatgactggcgccagacccacacgctgaaaaccctggccgattgggatgactggtgcgactttctgtattgtcgcacggttttctctgatatgaaactgaaagtcggctctaaacgtagtgatgacatcctggttcgtctgtttctgcgcgcactgacccagtgccaatggggtctgatgctgaaagataaaaaatcctactcatgtaaagaagtggcggaatggctgacctcggaaggctatagcgttaccgtcacggatgtcaaaaatgctgtgcgtgcgaaaattccgcagatgaaatttagctctgtgaccccgcgtatgaaatccctgatggacattatcgcccgtaaatatccgaccttttgcctgccggtttaactcgag

SEQ ID NO: 46 - protein, 4 aa, Escherichia coli
KTRG

SEQ ID NO: 47 - DNA, 50 bp, Artificial Sequence
  Oligonucleotide used for site-directed mutagenesis of the D368A variant
ccccgtcagatcactggtatgattacgccctggcaggcgcttataccacg

SEQ ID NO: 48 - DNA, 50 bp, Artificial Sequence
  Oligonucleotide used for site-directed mutagenesis of the D368A variant
gctggtataagcgcctgccagggcgtaatcataccagtgatctgacgggg

SEQ ID NO: 49 - DNA, 48 bp, Artificial Sequence
  Oligonucleotide used for site-directed mutagenesis of the D59A/E61A variant
ccctgcatatcggttttgccacggcatacgtgttcaacccggaaaccc

SEQ ID NO: 50 - DNA, 48 bp, Artificial Sequence
  Oligonucleotide used for site-directed mutagenesis of the D59A/E61A variant
gggtttccgggttgaacacgtatgccgtggcaaaaccgatatgcaggg

SEQ ID NO: 51 - DNA, 44 bp, Artificial Sequence
  Oligonucleotide used for site-directed mutagenesis of the WTHis variant
ccttttgcctgccggttttactcgagcaccaccaccaccaccac

SEQ ID NO: 52 - DNA, 44 bp, Artificial Sequence
  Oligonucleotide used for site-directed mutagenesis of the WTHis variant
gtggtggtggtggtggtgctcgagtaaaaccggcaggcaaaagg

SEQ ID NO: 53 - DNA, 48 bp, Artificial Sequence
  Oligonucleotide used for site-directed mutagenesis of the K613A variant
gggttcatcgatgctgacctgtgcacatgaagtctctcaactgatcgc

SEQ ID NO: 54 - DNA, 48 bp, Artificial Sequence
  Oligonucleotide used for site-directed mutagenesis of the K613A variant
gcgatcagttgagagacttcatgtgcacaggtcagcatcgatgaaccc

SEQ ID NO: 55 - DNA, 48 bp, Artificial Sequence
  Oligonucleotide used for site-directed mutagenesis of the H614A variant
gggttcatcgatgctgacctgtaaagctgaagtctctcaactgatcgc

SEQ ID NO: 56 - DNA, 48 bp, Artificial Sequence
  Oligonucleotide used for site-directed mutagenesis of the H614A variant
gcgatcagttgagagacttcagctttacaggtcagcatcgatgaaccc

SEQ ID NO: 57 - DNA, 42 bp, Artificial Sequence
  Oligonucleotide used for site-directed mutagenesis of the K623A variant
gtctctcaactgatcgccatggcaacccgtggtcagctgacg

SEQ ID NO: 58 - DNA, 42 bp, Artificial Sequence
  Oligonucleotide used for site-directed mutagenesis of the K623A variant
cgtcagctgaccacgggttgccatggcgatcagttgagagac

SEQ ID NO: 59 - DNA, 50 bp, Artificial Sequence
  Oligonucleotide used for site-directed mutagenesis of the R625A variant
gtctctcaactgatcgccatgaaaaccgctggtcagctgacgtataaagc

SEQ ID NO: 60 - DNA, 50 bp, Artificial Sequence
  Oligonucleotide used for site-directed mutagenesis of the R625A variant
gctttatacgtcagctgaccagcggttttcatggcgatcagttgagagac

SEQ ID NO: 61 - DNA, 4 bp, Artificial Sequence
  Oligonucleotide P4
gatc

SEQ ID NO: 62 - DNA, 10 bp, Artificial Sequence
  Oligonucleotide P10
gactgcttac

SEQ ID NO: 63 - DNA, 15 bp, Artificial Sequence
  Oligonucleotide P15
gatcacagtgagtac

SEQ ID NO: 64 - DNA, 33 bp, Artificial Sequence
  Oligonucleotide T33GTA
actggccgtcgttctattgtactcactgtgatc

SEQ ID NO: 65 - DNA, 33 bp, Artificial Sequence
  Oligonucleotide T33GTT
actggccgtcgttctaatgtactcactgtgatc

SEQ ID NO: 66 - DNA, 33 bp, Artificial Sequence
  Oligonucleotide T33GFT
  misc_feature (18)..(18): THF abasic site analog (F)
actggccgtcgttctatngtactcactgtgatc

SEQ ID NO: 67 - DNA, 14 bp, Artificial Sequence
  Oligonucleotide P20-33
gaacgacggccagt

SEQ ID NO: 68 - DNA, 33 bp, Artificial Sequence
  Oligonucleotide  33A
aaaaaaaaaaaaaaaaaaaaaaaaaaaaaaaaa

SEQ ID NO: 69 - DNA, 33 bp, Artificial Sequence
  Oligonucleotide 33T*
ttttttttttttttttttttttttttttttttt

SEQ ID NO: 70 - DNA, 33 bp, Artificial Sequence
  Oligonucleotides CC31T*
ccttttttttttttttttttttttttttttttt

SEQ ID NO: 71 - DNA, 33 bp, Artificial Sequence
  Oligonucleotide 15TCC16T*
ttttttttttttttccttttttttttttttttt

SEQ ID NO: 72 - DNA, 33 bp, Artificial Sequence
  Oligonucleotide 15TC17T*
ttttttttttttttctttttttttttttttttt

SEQ ID NO: 73 - DNA, 33 bp, Artificial Sequence
  Oligonucleotide  15TA17T*
ttttttttttttttatttttttttttttttttt

SEQ ID NO: 74 - DNA, 17 bp, Artificial Sequence
  Oligonucleotide M13 UP
gtaaaacgacggccagt

SEQ ID NO: 75 - protein, 553 aa, Salmonella virus
MPRRSRKKVEYKIAAFDFETDPFKHDRIPKPFSWGFYNGEIYKDYWGDDCIEQFIYWLDTIEEPHVIYAHNGGKFDFLFLMKYFRGKLKIVNGRILEVEHGIHKFRDSYAILPVPLAASDEKIEIDYGKMERETREQHKAEILEYLKGDCVTLHKMVSLFIAEFGMRLTIGGTAMNELKQFHPYDPVRKGFDEAMRPFYFGGRCQAFEKGIIEDDIKVYDVNSMYPHAMRNFRHPFSDEFYEANEITEETYFIEWEGENNGAVPVRTKTGLDFNQRSGIFHTSIHEWRAGIDTGTIKPNRIIRTINFTETTTFGAFIDHFFSKRDAAKKAGDLFHNIFYKLILNSSYGKFAQNPENYKEWCITEGGIYLEGYDGEGCEVQEHLDYILWGRPAEMFNYFNVAVAASITGAARSVLLRALAQAERPLYCDTDSIICRDLKNVPLDAYQLGAWDLEATGDKIAIAGKKLYALYAGDNCVKIASKGASLVPRDIGFLMPPDMEPKAAKKVAQQKAKNIGGEKILKVANGGVYDFVNDAPSFKLNGNVQFIKRTIKGT

SEQ ID NO: 76 - protein, 568 aa, Streptococcus phage
MTCYYAGDFETTTNEEETEVWLSCFAKVIDYDKLDTFKVNTSLEDFLKSLYLDLDKTYTETGEDEFIIFFHNLKFDGSFLLSFFLNNDIECTYFINDMGVWYSITLEFPDFTLTFRDSLKILNFSIATMAGLFKMPIAKGTTPLLKHKPEVIKPEWIDYIHVDVAILARGIFAMYYEENFTKYTSASEALTEFKRIFRKSKRKFRDFFPILDEKVDDFCRKHIVGAGRLPTLKHRGRTLNQLIDIYDINSMYPATMLQNALPIGIPKRYKGKPKEIKEDHYYIYHIKADFDLKRGYLPTIQIKKKLDALRIGVRTSDYVTTSKNEVIDLYLTNFDLDLFLKHYDATIMYVETLEFQTESDLFDDYITTYRYKKENAQSPAEKQKAKIMLNSLYGKFGAKIISVKKLAYLDDKGILRFKNDDEEEVQPVYAPVALFVTSIARHFIISNAQENYDNFLYADTDSLHLFHSDSLVLDIDPSEFGKWAHEGRAVKAKYLRSKLYIEELIQEDGTTHLDVKGAGMTPEIKEKITFENFVIGATFEGKRASKQIKGGTLIYETTFKIRETDYLV

SEQ ID NO: 77 - protein, 717 aa, His 1 virus
MAKCDKSLEAIDLDRAYTAPRKAKWAENKRINGLDTETSDGDIFCISVCWEGEKPMVQHNDREKLTSKQVWQVLTDHKARSSLNMWYNLDFDANVVLNHVCSEEQLAELVVSGTTLANSDRTYRQYMDTDKELRKGEYLITYIQSKFLEIKDHNSHIYTHYDASQFFYTSLENAVTEWLGESKANDGLEAGLFGSQTPNQLRETVAESDCVTWTNLSLTYNVSKGDKWTIHNAKSYISKNWSDILKYAQIDAELVRDLWQEAVNVGEELDIPMGRPFSTGYLAESYLDNRLREKPGLGPMPMAKMAWESYAGGRFEVLKRGNVGRVAGPDINSAYPAVLAELPDPKTLRWKRAKHASISEIETADYGFMTVKVSTDPTREIQPFAVKDEKQDKLVYPSPQNTEITVVKDIFIHAYNQGYVTDYEVIDCWLGYKTEGTTFPFDFIPELYDNRKTAEANGLEKRGLLLKIVLNSMYGKTCQTTPKRRELAESTELELHESYVPDMSLPKMIREKYSEGFIESLTAGAWFNPFLASYITGLTRLELHKQICKHDLEENTVMLATDCVMIEEKPFEESNFVENLVQDGLGYWDMEYKGDAFVLGAGVYQIDFDTCQKGCKDNCNKFSHKHKVKTRGFSEADLEKGLVNAAEKANGHIEIESTRPQTISEIIWSNEELSQVGNFLEQERKIKPEMDTKRKWSENTDFKKLLSTCETSLPLKI

SEQ ID NO: 78 - protein, 720 aa, His2 virus
MAKSDRNLDEVNLYPAYQDQYSATFVDGKLINAFDTETSSGTVFMLTSAYGDKTQAYYNRDVSELDAETIMDALTDYKTRSNINIWYNLDFDANAILSGILSQKEMSELVVTNETTTTVAGIEYEIFYIKGKMLRIVDENGNISPHYDIAQFFYTSLDNAAEEWLGENKKEGIDTSKFDDKEYIKDNFDEILKYAKKDASLTQDLAIELTNEAENLDIPMGRPISTGYLSAEYLRANTEEKPSLGNEAMQNLFWESYYGGRFEVFQRGNVGEVVAPDINSAYPAIMKDLPDPTTLNWNHYLNEVSDKEPFSHSINKFGYEEIENGHYGVVKARVTTDSSRMIQPFACKIDGKVKFPAMTNKVVTVIKPIFEFAVNNGLVTDFELIEAWIGNITDRTSKPFEFIGDMYAERKVFEQLKNKPKKGQLLKIVLNSSYGKTCQTTEKRHKHDLDKDGKKIMQAHETQYPRFYLSKKQREALGDDEIIITELEAGKRFNPFFASYITGLTRLELHKQVVEHDIEDSTVMFATDCLMVEKEAYENSSFDEQIHVPDDSLPESEFRKEATRSLGAWDFDYEGSAFIVGSGVYEVDTIQGKTKTKTRGFIESNLGDTLKGLAKKHKEAIPLDNERPLTMAEVLINTERGSVSEFVENSKKLKPDFDDKRNWNRENPNFHDLLNDKEYSKPIDLQEQKEEMIQEQMDINEKMIGDATPNGNETVVVKDD

SEQ ID NO: 79 - DNA, 33 bp, Artificial Sequence; identical to SEQ ID NO: 64
  Oligonucleotide template substrate used in the examples

SEQ ID NO: 80 - DNA, 33 bp, Artificial Sequence; identical to SEQ ID NO: 65
  Oligonucleotide template substrate used in the examples

SEQ ID NO: 81 - DNA, 33 bp, Artificial Sequence; identical to SEQ ID NO: 66
  Oligonucleotide template substrate used in the examples
  misc_feature (18)..(18): THF abasic site analog (F)

SEQ ID NO: 82 - DNA, 33 bp, Artificial Sequence
  Oligonucleotide template substrate used in the examples
  misc_feature (18)..(18): THF abasic site analog (F)
actggccgtcgttctaangtactcactgtgatc

SEQ ID NO: 83 - DNA, 33 bp, Artificial Sequence; identical to SEQ ID NO: 66
  Oligonucleotide template substrate used in the examples
  misc_feature (18)..(18): T, THF, Tg or T:T

SEQ ID NO: 84 - DNA, 33 bp, Artificial Sequence; identical to SEQ ID NO: 82
  Oligonucleotide template substrate used in the examples
  misc_feature (18)..(18): T or THF

SEQ ID NO: 85 - protein, 14 aa, Artificial Sequence
  SEQ ID NO: 1 in which X2 is H and X3-10 is SEQ ID NO: 5
KHEVSQLIAMKTRG